European Patent Application EP 4 497 826 A1, published January 29, 2025. Title: ＴＤＰ－４３の凝集抑制剤及び医薬組成物. Applicant: Niigata University. The sequence listing filed with the application follows.

SEQUENCE LISTING (21 sequences)

SEQ ID NO: 1 - protein, 414 aa, Homo sapiens
MSEYIRVTEDENDEPIEIPSEDDGTVLLSTVTAQFPGACGLRYRNPVSQCMRGVRLVEGILHAPDAGWGNLVYVVNYPKDNKRKMDETDASSAVKVKRAVQKTSDLIVLGLPWKTTEQDLKEYFSTFGEVLMVQVKKDLKTGHSKGFGFVRFTEYETQVKVMSQRHMIDGRWCDCKLPNSKQSQDEPLRSRKVFVGRCTEDMTEDELREFFSQYGDVMDVFIPKPFRAFAFVTFADDQIAQSLCGEDLIIKGISVHISNAEPKHNSNRQLERSGRFGGNPGGFGNQGGFGNSRGGGAGLGNNQGSNMGGGMNFGAFSINPAMMAAAQAALQSSWGMMGMLASQQNQSGPSGNNQNQGNMQREPNQAFGSGNNSYSGSNSGAAIGWGSASNAGSGSGFNGGFGSSMDSKSSGWGM

SEQ ID NO: 2 - protein, 295 aa, Homo sapiens
MSEYIRVTEDENDEPIEIPSEDDGTVLLSTVTAQFPGACGLRYRNPVSQCMRGVRLVEGILHAPDAGWGNLVYVVNYPKDNKRKMDETDASSAVKVKRAVQKTSDLIVLGLPWKTTEQDLKEYFSTFGEVLMVQVKKDLKTGHSKGFGFVRFTEYETQVKVMSQRHMIDGRWCDCKLPNSKQSQDEPLRSRKVFVGRCTEDMTEDELREFFSQYGDVMDVFIPKPFRAFAFVTFADDQIAQSLCGEDLIIKGISVHISNAEPKHNSNRQLERSGRFGVHLISNVYGRSTSLKVVL

SEQ ID NO: 3 - protein, 238 aa, Homo sapiens
MSEYIRVTEDENDEPIEIPSEDDGTVLLSTVTAQFPGACGLRYRNPVSQCMRGVRLVEGILHAPDAGWGNLVYVVNYPKDNKRKMDETDASSAVKVKRAVQKTSDLIVLGLPWKTTEQDLKEYFSTFGEVLMVQVKKDLKTGHSKGFGFVRFTEYETQVKVMSQRHMIDGRWCDCKLPNSKQSQDEPLRSRKVFVGRCTEDMTEDELREFFSQYGDVMDVFIPKPFRAFAFVTFADDQ

SEQ ID NO: 4 - DNA, 888 bp, Homo sapiens
  source 1..888: mol_type = other DNA
atgtctgaatatattcgggtaaccgaagatgagaacgatgagcccattgaaataccatcggaagacgatgggacggtgctgctctccacggttacagcccagtttccaggggcgtgtgggcttcgctacaggaatccagtgtctcagtgtatgagaggtgtccggctggtagaaggaattctgcatgccccagatgctggctggggaaatctggtgtatgttgtcaactatccaaaagataacaaaagaaaaatggatgagacagatgcttcatcagcagtgaaagtgaaaagagcagtccagaaaacatccgatttaatagtgttgggtctcccatggaaaacaaccgaacaggacctgaaagagtattttagtacctttggagaagttcttatggtgcaggtcaagaaagatcttaagactggtcattcaaaggggtttggctttgttcgttttacggaatatgaaacacaagtgaaagtaatgtcacagcgacatatgatagatggacgatggtgtgactgcaaacttcctaattctaagcaaagccaagatgagcctttgagaagcagaaaagtgtttgtggggcgctgtacagaggacatgactgaggatgagctgcgggagttcttctctcagtacggggatgtgatggatgtcttcatccccaagccattcagggcctttgcctttgttacatttgcagatgatcagattgcgcagtctctttgtggagaggacttgatcattaaaggaatcagcgttcatatatccaatgccgaacctaagcacaatagcaatagacagttagaaagaagtggaagatttggtgttcatctcatttcaaatgtttatggaagaagcacttcattgaaagtagtgctgtaa

SEQ ID NO: 5 - DNA, 714 bp, Homo sapiens
  source 1..714: mol_type = other DNA
atgtctgaatatattcgggtaaccgaagatgagaacgatgagcccattgaaataccatcggaagacgatgggacggtgctgctctccacggttacagcccagtttccaggggcgtgtgggcttcgctacaggaatccagtgtctcagtgtatgagaggtgtccggctggtagaaggaattctgcatgccccagatgctggctggggaaatctggtgtatgttgtcaactatccaaaagataacaaaagaaaaatggatgagacagatgcttcatcagcagtgaaagtgaaaagagcagtccagaaaacatccgatttaatagtgttgggtctcccatggaaaacaaccgaacaggacctgaaagagtattttagtacctttggagaagttcttatggtgcaggtcaagaaagatcttaagactggtcattcaaaggggtttggctttgttcgttttacggaatatgaaacacaagtgaaagtaatgtcacagcgacatatgatagatggacgatggtgtgactgcaaacttcctaattctaagcaaagccaagatgagcctttgagaagcagaaaagtgtttgtggggcgctgtacagaggacatgactgaggatgagctgcgggagttcttctctcagtacggggatgtgatggatgtcttcatccccaagccattcagggcctttgcctttgttacatttgcagatgatcag

SEQ ID NO: 6 - DNA, 1837 bp, synthetic construct
  misc_feature 1..1837: note = synthesized nucleotides
  source 1..1837: mol_type = other DNA
atgtctgaatatattcgggtaaccgaagatgagaacgatgagcccattgaaataccatcggaagacgatgggacggtgctgctctccacggttacagcccagtttccaggggcgtgtgggcttcgctacaggaatccagtgtctcagtgtatgagaggtgtccggctggtagaaggaattctgcatgccccagatgctggctggggaaatctggtgtatgttgtcaactatccaaaagataacaaaagaaaaatggatgagacagatgcttcatcagcagtgaaagtgaaaagagcagtccagaaaacatccgatttaatagtgttgggtctcccatggaaaacaaccgaacaggacctgaaagagtattttagtacctttggagaagttcttatggtgcaggtcaagaaagatcttaagactggtcattcaaaggggtttggctttgttcgttttacggaatatgaaacacaagtgaaagtaatgtcacagcgacatatgatagatggacgatggtgtgactgcaaacttcctaattctaagcaaagccaagatgagcctttgagaagcagaaaagtgtttgtggggcgctgtacagaggacatgactgaggatgagctgcgggagttcttctctcagtacggggatgtgatggatgtcttcatccccaagccattcagggcctttgcctttgttacatttgcagatgatcagattgcgcagtctctttgtggagaggacttgatcattaaaggaatcagcgttcatatatccaatgccgaacctaagcacaatagcaatagacagttagaaagaagtggaagatttggtgttcatctcatttcaaatgtttatggaagaagcacttcattgaaagtagtgctgtaaatattctgccataggaatactgtctacatgctttctcattcaagaattcgtcatcacgcatcacaggccgcgtctttgacggtgggtgtcccatttttatccgctactctttatttcatggagtcgtatcaacgctatgaacgcaaggctgtgatatggaaccagaaggctgtctgaacttttgaaaccttgtgtgtgtgtgtgtgtgggattgatggtggtgccgaggcatgaaaggctagtatgagcgagaaaaggagagagcgcgtgcagagacttggtggtgcataatggatattttttaacttggcgagatgtgtctctcaatcctgtggctttggtgagagagtgtgcagagagcaatgatagcaaataatgtacgaatgttttttgcattcaaaggacatccacatctgttggaagacttttaagtgagtttttgttcttagataacccacattagatgaatgtgttaagtgaaatgatacttgtactccccctacccctttgtcaactgctgtgaatgctgtatggtgtgtgtgtgtgtgttctcttctgttactgatatgtaagtgtggcaatgtgaactgaagctgatgggctgagaacatggactgagcttgtggtgtgctttgcaggaggacttgaagcagagttcaccagtgagctcaggtgtctcaaagaagggtggaagttctaatgtctgttagctacccataagaatgctgtttgctgcagttctgtgtcctgtgcttggatgctttttataagagttgtcattgttggaaattcttaaataaaactgatttaaataatatgtgtctttgttttgcagccctgaatgcaaagaattcatagcagttaattccccttttttgacccttttgagatggaactttcataaagtttcttggcagtagtttattttgcttcaaataaacttatttga

SEQ ID NO: 7 - DNA, 4185 bp, Homo sapiens
  source 1..4185: mol_type = other DNA
attttgtgggagcgaagcggtggctgggctgcgcttgggtccgtcgctgcttcggtgtccctgtcgggcttcccagcagcggcctagcgggaaaagtaaaagatgtctgaatatattcgggtaaccgaagatgagaacgatgagcccattgaaataccatcggaagacgatgggacggtgctgctctccacggttacagcccagtttccaggggcgtgtgggcttcgctacaggaatccagtgtctcagtgtatgagaggtgtccggctggtagaaggaattctgcatgccccagatgctggctggggaaatctggtgtatgttgtcaactatccaaaagataacaaaagaaaaatggatgagacagatgcttcatcagcagtgaaagtgaaaagagcagtccagaaaacatccgatttaatagtgttgggtctcccatggaaaacaaccgaacaggacctgaaagagtattttagtacctttggagaagttcttatggtgcaggtcaagaaagatcttaagactggtcattcaaaggggtttggctttgttcgttttacggaatatgaaacacaagtgaaagtaatgtcacagcgacatatgatagatggacgatggtgtgactgcaaacttcctaattctaagcaaagccaagatgagcctttgagaagcagaaaagtgtttgtggggcgctgtacagaggacatgactgaggatgagctgcgggagttcttctctcagtacggggatgtgatggatgtcttcatccccaagccattcagggcctttgcctttgttacatttgcagatgatcagattgcgcagtctctttgtggagaggacttgatcattaaaggaatcagcgttcatatatccaatgccgaacctaagcacaatagcaatagacagttagaaagaagtggaagatttggtggtaatccaggtggctttgggaatcagggtggatttggtaatagcagagggggtggagctggtttgggaaacaatcaaggtagtaatatgggtggtgggatgaactttggtgcgttcagcattaatccagccatgatggctgccgcccaggcagcactacagagcagttggggtatgatgggcatgttagccagccagcagaaccagtcaggcccatcgggtaataaccaaaaccaaggcaacatgcagagggagccaaaccaggccttcggttctggaaataactcttatagtggctctaattctggtgcagcaattggttggggatcagcatccaatgcagggtcgggcagtggttttaatggaggctttggctcaagcatggattctaagtcttctggctggggaatgtagacagtggggttgtggttggttggtatagaatggtgggaattcaaatttttctaaactcatggtaagtatattgtaaaatacatatgtactaagaattttcaaaattggtttgttcagtgtggagtatattcagcagtatttttgacatttttctttagaaaaaggaagagctaaaggaattttataagttttgttacatgaaaggttgaaatattgagtggttgaaagtgaactgctgtttgcctgattggtaaaccaacacactacaattgatatcaaaaggtttctcctgtaatattttatccctggacttgtcaagtgaattctttgcatgttcaaaacggaaaccattgattagaactacattctttaccccttgttttaatttgaaccccaccatatggatttttttccttaagaaaatctccttttaggagatcatggtgtcacagtgtttggttcttttgttttgttttttaacacttgtctcccctcatacacaaaagtacaatatgaagccttcatttaatctctgcagttcatctcatttcaaatgtttatggaagaagcacttcattgaaagtagtgctgtaaatattctgccataggaatactgtctacatgctttctcattcaagaattcgtcatcacgcatcacaggccgcgtctttgacggtgggtgtcccatttttatccgctactctttatttcatggagtcgtatcaacgctatgaacgcaaggctgtgatatggaaccagaaggctgtctgaacttttgaaaccttgtgtgggattgatggtggtgccgaggcatgaaaggctagtatgagcgagaaaaggagagagcgcgtgcagagacttggtggtgcataatggatattttttaacttggcgagatgtgtctctcaatcctgtggctttggtgagagagtgtgcagagagcaatgatagcaaataatgtacgaatgttttttgcattcaaaggacatccacatctgttggaagacttttaagtgagtttttgttcttagataacccacattagatgaatgtgttaagtgaaatgatacttgtactccccctacccctttgtcaactgctgtgaatgctgtatggtgtgtgttctcttctgttactgatatgtaagtgtggcaatgtgaactgaagctgatgggctgagaacatggactgagcttgtggtgtgctttgcaggaggacttgaagcagagttcaccagtgagctcaggtgtctcaaagaagggtggaagttctaatgtctgttagctacccataagaatgctgtttgctgcagttctgtgtcctgtgcttggatgctttttataagagttgtcattgttggaaattcttaaataaaactgatttaaataatatgtgtctttgttttgcagccctgaatgcaaagaattcatagcagttaattccccttttttgacccttttgagatggaactttcataaagtttcttggcagtagtttattttgcttcaaataaacttatttgaaaagttgtctcaagtcaaatggattcatcacctgtcatgcattgacacctgatacccagacttaattggtatttgttcttgcattggccaaagtgaaaatttttttttttcttttgaaatctagttttgaataagtctgggtgaccgcacctaaaatggtaagcagtaccctccggctttttcttagtgcctctgtgcatttgggtgatgttctatttacatggcctgtgtaaatctccattgggaagtcatgccttctaaaaagattcttatttgggggagtgggcaaaatgttgattattttctaatgctttgtagcaaagcatatcaattgaaaagggaatatcagcaccttcctagtttgggatttgaaaagtggaattaattgcagtagggataaagtagaagaaaccacaaattatcttgtgcctgaaatccattaagaggcctgatagctttaagaattagggtgggttgtctgtctggaagtgttaagtggaatgggctttgtcctccaggaggtgggggaatgtggtaacattgaatacagttgaataaaatcgcttacaaaactcacactctcacaatgcattgttaagtatgtaaaagcaataacattgattctctgttgtacttttttgtaactaattctgtgagagttgagctcattttctagttggaagaatgtgatatttgttgtgttggtagtttacctaatgcccttacctaattagattatgataaataggtttgtcattttgcaagttacataaacatttatcaatgaagtcatcctttagacttgtaatcgccacattgtttcattattcagtttcctctgtaaagggatcttgagttgttttaattttttttttctgcatctgaatctgcatgatttccaaaccctgtaccatctgaattttgcattttagcacttgcactattactcagcagcagtaacatggtaacacttaaaatggtactcggggacctccaaagactaaactgacaagccttcaaggagcccaggggtaagttaacttgtcaacggcatggtttaatcccttctttacacttgtgtaaatttcagttactggtcatagaaggctttcaatgttgagtggccttttattaacatgtttatggtactgcatagatacgggtatttattttaccctaagaagattttgaagtttaaaagtacttaaactatttggcaaagatttgtttttaaaaatctatttggtcaatctaaatgcattcattctaaaaaattttttgaaccagataaataaaatttttttttgacaccaca

SEQ ID NO: 8 - DNA, 12 bp, synthetic construct
  misc_feature 1..12: note = Synthesized nucleotides
  source 1..12: mol_type = other DNA
tgtgtgtgtgtg

SEQ ID NO: 9 - skipped

SEQ ID NO: 10 - DNA, 949 bp, synthetic construct
  misc_feature 1..949: note = Synthesized nucleotides
  source 1..949: mol_type = other DNA
atattctgccataggaatactgtctacatgctttctcattcaagaattcgtcatcacgcatcacaggccgcgtctttgacggtgggtgtcccatttttatccgctactctttatttcatggagtcgtatcaacgctatgaacgcaaggctgtgatatggaaccagaaggctgtctgaacttttgaaaccttgtgtgtgtgtgtgtgtgggattgatggtggtgccgaggcatgaaaggctagtatgagcgagaaaaggagagagcgcgtgcagagacttggtggtgcataatggatattttttaacttggcgagatgtgtctctcaatcctgtggctttggtgagagagtgtgcagagagcaatgatagcaaataatgtacgaatgttttttgcattcaaaggacatccacatctgttggaagacttttaagtgagtttttgttcttagataacccacattagatgaatgtgttaagtgaaatgatacttgtactccccctacccctttgtcaactgctgtgaatgctgtatggtgtgtgtgtgtgtgttctcttctgttactgatatgtaagtgtggcaatgtgaactgaagctgatgggctgagaacatggactgagcttgtggtgtgctttgcaggaggacttgaagcagagttcaccagtgagctcaggtgtctcaaagaagggtggaagttctaatgtctgttagctacccataagaatgctgtttgctgcagttctgtgtcctgtgcttggatgctttttataagagttgtcattgttggaaattcttaaataaaactgatttaaataatatgtgtctttgttttgcagccctgaatgcaaagaattcatagcagttaattccccttttttgacccttttgagatggaactttcataaagtttcttggcagtagtttattttgcttcaaataaacttatttga

SEQ ID NO: 11 - protein, 215 aa, synthetic construct
  REGION 1..215: note = synthesized polypeptide
NKRKMDETDASSAVKVKRAVQKTSDLIVLGLPWKTTEQDLKEYFSTFGEVLMVQVKKDLKTGHSKGFGFVRFTEYETQVKVMSQRHMIDGRWCDCKLPNSKQSQDEPLRSRKVFVGRCTEDMTEDELREFFSQYGDVMDVFIPKPFRAFAFVTFADDQIAQSLCGEDLIIKGISVHISNAEPKHNSNRQLERSGRFGVHLISNVYGRSTSLKVVL

SEQ ID NO: 12 - DNA, 2133 bp, synthetic construct
  misc_feature 1..2133: note = synthesized nucleotides
  source 1..2133: mol_type = other DNA
atgtctgaatatattcgggtaaccgaagatgagaacgatgagcccattgaaataccatcggaagacgatgggacggtgctgctctccacggttacagcccagtttccaggggcgtgtgggcttcgctacaggaatccagtgtctcagtgtatgagaggtgtccggctggtagaaggaattctgcatgccccagatgctggctggggaaatctggtgtatgttgtcaactatccaaaagataacaaaagaaaaatggatgagacagatgcttcatcagcagtgaaagtgaaaagagcagtccagaaaacatccgatttaatagtgttgggtctcccatggaaaacaaccgaacaggacctgaaagagtattttagtacctttggagaagttcttatggtgcaggtcaagaaagatcttaagactggtcattcaaaggggtttggctttgttcgttttacggaatatgaaacacaagtgaaagtaatgtcacagcgacatatgatagatggacgatggtgtgactgcaaacttcctaattctaagcaaagccaagatgagcctttgagaagcagaaaagtgtttgtggggcgctgtacagaggacatgactgaggatgagctgcgggagttcttctctcagtacggggatgtgatggatgtcttcatccccaagccattcagggcctttgcctttgttacatttgcagatgatcagattgcgcagtctctttgtggagaggacttgatcattaaaggaatcagcgttcatatatccaatgccgaacctaagcacaatagcaatagacagttagaaagaagtggaagatttggtggtaatccaggtggctttgggaatcagggtggatttggtaatagcagagggggtggagctggtttgggaaacaatcaaggtagtaatatgggtggtgggatgaactttggtgcgttcagcattaatccagccatgatggctgccgcccaggcagcactacagagcagttggggtatgatgggcatgttagccagccagcagaaccagtcaggcccatcgggtaataaccaaaaccaaggcaacatgcagagggagccaaaccaggccttcggttctggaaataactcttatagtggctctaattctggtgcagcaattggttggggatcagcatccaatgcagggtcgggcagtggttttaatggaggctttggctcaagcatggattctaagtcttctggctggggaatggcagaaatcggtactggctttccattcgacccccattatgtggaagtcctgggcgagcgcatgcactacgtcgatgttggtccgcgcgatggcacccctgtgctgttcctgcacggtaacccgacctcctcctacgtgtggcgcaacatcatcccgcatgttgcaccgacccatcgctgcattgctccagacctgatcggtatgggcaaatccgacaaaccagacctgggttatttcttcgacgaccacgtccgcttcatggatgccttcatcgaagccctgggtctggaagaggtcgtcctggtcattcacgactggggctccgctctgggtttccactgggccaagcgcaatccagagcgcgtcaaaggtattgcatttatggagttcatccgccctatcccgacctgggacgaatggccagaatttgcccgcgagaccttccaggccttccgcaccaccgacgtcggccgcaagctgatcatcgatcagaacgtttttatcgagggtacgctgccgatgggtgtcgtccgcccgctgactgaagtcgagatggaccattaccgcgagccgttcctgaatcctgttgaccgcgagccactgtggcgcttcccaaacgagctgccaatcgccggtgagccagcgaacatcgtcgcgctggtcgaagaatacatggactggctgcaccagtcccctgtcccgaagctgctgttctggggcaccccaggcgttctgatcccaccggccgaagccgctcgcctggccaaaagcctgcctaactgcaaggctgtggacatcggcccgggtctgaatctgctgcaagaagacaacccggacctgatcggcagcgagatcgcgcgctggctgtcgacgctcgagatttccggctag

SEQ ID NO: 13 - DNA, 1776 bp, synthetic construct
  misc_feature 1..1776: note = synthesized nucleotides
  source 1..1776: mol_type = other DNA
atgtctgaatatattcgggtaaccgaagatgagaacgatgagcccattgaaataccatcggaagacgatgggacggtgctgctctccacggttacagcccagtttccaggggcgtgtgggcttcgctacaggaatccagtgtctcagtgtatgagaggtgtccggctggtagaaggaattctgcatgccccagatgctggctggggaaatctggtgtatgttgtcaactatccaaaagataacaaaagaaaaatggatgagacagatgcttcatcagcagtgaaagtgaaaagagcagtccagaaaacatccgatttaatagtgttgggtctcccatggaaaacaaccgaacaggacctgaaagagtattttagtacctttggagaagttcttatggtgcaggtcaagaaagatcttaagactggtcattcaaaggggtttggctttgttcgttttacggaatatgaaacacaagtgaaagtaatgtcacagcgacatatgatagatggacgatggtgtgactgcaaacttcctaattctaagcaaagccaagatgagcctttgagaagcagaaaagtgtttgtggggcgctgtacagaggacatgactgaggatgagctgcgggagttcttctctcagtacggggatgtgatggatgtcttcatccccaagccattcagggcctttgcctttgttacatttgcagatgatcagattgcgcagtctctttgtggagaggacttgatcattaaaggaatcagcgttcatatatccaatgccgaacctaagcacaatagcaatagacagttagaaagaagtggaagatttggtgttcatctcatttcaaatgtttatggaagaagcacttcattgaaagtagtgctggcagaaatcggtactggctttccattcgacccccattatgtggaagtcctgggcgagcgcatgcactacgtcgatgttggtccgcgcgatggcacccctgtgctgttcctgcacggtaacccgacctcctcctacgtgtggcgcaacatcatcccgcatgttgcaccgacccatcgctgcattgctccagacctgatcggtatgggcaaatccgacaaaccagacctgggttatttcttcgacgaccacgtccgcttcatggatgccttcatcgaagccctgggtctggaagaggtcgtcctggtcattcacgactggggctccgctctgggtttccactgggccaagcgcaatccagagcgcgtcaaaggtattgcatttatggagttcatccgccctatcccgacctgggacgaatggccagaatttgcccgcgagaccttccaggccttccgcaccaccgacgtcggccgcaagctgatcatcgatcagaacgtttttatcgagggtacgctgccgatgggtgtcgtccgcccgctgactgaagtcgagatggaccattaccgcgagccgttcctgaatcctgttgaccgcgagccactgtggcgcttcccaaacgagctgccaatcgccggtgagccagcgaacatcgtcgcgctggtcgaagaatacatggactggctgcaccagtcccctgtcccgaagctgctgttctggggcaccccaggcgttctgatcccaccggccgaagccgctcgcctggccaaaagcctgcctaactgcaaggctgtggacatcggcccgggtctgaatctgctgcaagaagacaacccggacctgatcggcagcgagatcgcgcgctggctgtcgacgctcgagatttccggctag

SEQ ID NO: 14 - DNA, 1536 bp, synthetic construct
  misc_feature 1..1536: note = synthesized nucleotides
  source 1..1536: mol_type = other DNA
aacaaaagaaaaatggatgagacagatgcttcatcagcagtgaaagtgaaaagagcagtccagaaaacatccgatttaatagtgttgggtctcccatggaaaacaaccgaacaggacctgaaagagtattttagtacctttggagaagttcttatggtgcaggtcaagaaagatcttaagactggtcattcaaaggggtttggctttgttcgttttacggaatatgaaacacaagtgaaagtaatgtcacagcgacatatgatagatggacgatggtgtgactgcaaacttcctaattctaagcaaagccaagatgagcctttgagaagcagaaaagtgtttgtggggcgctgtacagaggacatgactgaggatgagctgcgggagttcttctctcagtacggggatgtgatggatgtcttcatccccaagccattcagggcctttgcctttgttacatttgcagatgatcagattgcgcagtctctttgtggagaggacttgatcattaaaggaatcagcgttcatatatccaatgccgaacctaagcacaatagcaatagacagttagaaagaagtggaagatttggtgttcatctcatttcaaatgtttatggaagaagcacttcattgaaagtagtgctggcagaaatcggtactggctttccattcgacccccattatgtggaagtcctgggcgagcgcatgcactacgtcgatgttggtccgcgcgatggcacccctgtgctgttcctgcacggtaacccgacctcctcctacgtgtggcgcaacatcatcccgcatgttgcaccgacccatcgctgcattgctccagacctgatcggtatgggcaaatccgacaaaccagacctgggttatttcttcgacgaccacgtccgcttcatggatgccttcatcgaagccctgggtctggaagaggtcgtcctggtcattcacgactggggctccgctctgggtttccactgggccaagcgcaatccagagcgcgtcaaaggtattgcatttatggagttcatccgccctatcccgacctgggacgaatggccagaatttgcccgcgagaccttccaggccttccgcaccaccgacgtcggccgcaagctgatcatcgatcagaacgtttttatcgagggtacgctgccgatgggtgtcgtccgcccgctgactgaagtcgagatggaccattaccgcgagccgttcctgaatcctgttgaccgcgagccactgtggcgcttcccaaacgagctgccaatcgccggtgagccagcgaacatcgtcgcgctggtcgaagaatacatggactggctgcaccagtcccctgtcccgaagctgctgttctggggcaccccaggcgttctgatcccaccggccgaagccgctcgcctggccaaaagcctgcctaactgcaaggctgtggacatcggcccgggtctgaatctgctgcaagaagacaacccggacctgatcggcagcgagatcgcgcgctggctgtcgacgctcgagatttccggctag

SEQ ID NO: 15-16 - skipped (2 entries)

SEQ ID NO: 17 - DNA, 1850 bp, synthetic construct
  misc_feature 1..1850: note = Synthesized nucleotides
  source 1..1850: mol_type = other DNA
atggaacaaaaactcatctcagaagaggatctgatgtctgaatatattcgggtaaccgaagatgagaacgatgagcccattgaaataccatcggaagacgatgggacggtgctgctctccacggttacagcccagtttccaggggcgtgtgggcttcgctacaggaatccagtgtctcagtgtatgagaggtgtccggctggtagaaggaattctgcatgccccagatgctggctggggaaatctggtgtatgttgtcaactatccaaaagataacaaaagaaaaatggatgagacagatgcttcatcagcagtgaaagtgaaaagagcagtccagaaaacatccgatttaatagtgttgggtctcccatggaaaacaaccgaacaggacctgaaagagtattttagtacctttggagaagttcttatggtgcaggtcaagaaagatcttaagactggtcattcaaaggggtttggctttgttcgttttacggaatatgaaacacaagtgaaagtaatgtcacagcgacatatgatagatggacgatggtgtgactgcaaacttcctaattctaagcaaagccaagatgagcctttgagaagcagaaaagtgtttgtggggcgctgtacagaggacatgactgaggatgagctgcgggagttcttctctcagtacggggatgtgatggatgtcttcatccccaagccattcagggcctttgcctttgttacatttgcagatgatcagattgcgcagtctctttgtggagaggacttgatcattaaaggaatcagcgttcatatatccaatgccgaacctaagcacaatagcaatagacagttagaaagaagtggaagatttggtgttcatctcatttcaaatgtttatggaagaagcacttcattgaaagtagtgctgtaaatattctgccataggaatactgtctacatgctttctcattcaagaattcgtcatcacgcatcacaggccgcgtctttgacggtgggtgtcccatttttatccgctactctttatttcatggagtcgtatcaacgctatgaacgcaaggctgtgatatggaaccagaaggctgtctgaacttttgaaaccttgtgtgggattgatggtggtgccgaggcatgaaaggctagtatgagcgagaaaaggagagagcgcgtgcagagacttggtggtgcataatggatattttttaacttggcgagatgtgtctctcaatcctgtggctttggtgagagagtgtgcagagagcaatgatagcaaataatgtacgaatgttttttgcattcaaaggacatccacatctgttggaagacttttaagtgagtttttgttcttagataacccacattagatgaatgtgttaagtgaaatgatacttgtactccccctacccctttgtcaactgctgtgaatgctgtatggtgtgtgttctcttctgttactgatatgtaagtgtggcaatgtgaactgaagctgatgggctgagaacatggactgagcttgtggtgtgctttgcaggaggacttgaagcagagttcaccagtgagctcaggtgtctcaaagaagggtggaagttctaatgtctgttagctacccataagaatgctgtttgctgcagttctgtgtcctgtgcttggatgctttttataagagttgtcattgttggaaattcttaaataaaactgatttaaataatatgtgtctttgttttgcagccctgaatgcaaagaattcatagcagttaattccccttttttgacccttttgagatggaactttcataaagtttcttggcagtagtttattttgcttcaaataaacttatttga

SEQ ID NO: 18 - DNA, 1870 bp, synthetic construct
  misc_feature 1..1870: note = Synthesized nucleotides
  source 1..1870: mol_type = other DNA
atggaacaaaaactcatctcagaagaggatctgatgtctgaatatattcgggtaaccgaagatgagaacgatgagcccattgaaataccatcggaagacgatgggacggtgctgctctccacggttacagcccagtttccaggggcgtgtgggcttcgctacaggaatccagtgtctcagtgtatgagaggtgtccggctggtagaaggaattctgcatgccccagatgctggctggggaaatctggtgtatgttgtcaactatccaaaagataacaaaagaaaaatggatgagacagatgcttcatcagcagtgaaagtgaaaagagcagtccagaaaacatccgatttaatagtgttgggtctcccatggaaaacaaccgaacaggacctgaaagagtattttagtacctttggagaagttcttatggtgcaggtcaagaaagatcttaagactggtcattcaaaggggtttggctttgttcgttttacggaatatgaaacacaagtgaaagtaatgtcacagcgacatatgatagatggacgatggtgtgactgcaaacttcctaattctaagcaaagccaagatgagcctttgagaagcagaaaagtgtttgtggggcgctgtacagaggacatgactgaggatgagctgcgggagttcttctctcagtacggggatgtgatggatgtcttcatccccaagccattcagggcctttgcctttgttacatttgcagatgatcagattgcgcagtctctttgtggagaggacttgatcattaaaggaatcagcgttcatatatccaatgccgaacctaagcacaatagcaatagacagttagaaagaagtggaagatttggtgttcatctcatttcaaatgtttatggaagaagcacttcattgaaagtagtgctgtaaatattctgccataggaatactgtctacatgctttctcattcaagaattcgtcatcacgcatcacaggccgcgtctttgacggtgggtgtcccatttttatccgctactctttatttcatggagtcgtatcaacgctatgaacgcaaggctgtgatatggaaccagaaggctgtctgaacttttgaaaccttgtgtgtgtgtgtgtgtgggattgatggtggtgccgaggcatgaaaggctagtatgagcgagaaaaggagagagcgcgtgcagagacttggtggtgcataatggatattttttaacttggcgagatgtgtctctcaatcctgtggctttggtgagagagtgtgcagagagcaatgatagcaaataatgtacgaatgttttttgcattcaaaggacatccacatctgttggaagacttttaagtgagtttttgttcttagataacccacattagatgaatgtgttaagtgaaatgatacttgtactccccctacccctttgtcaactgctgtgaatgctgtatggtgtgtgtgtgtgtgttctcttctgttactgatatgtaagtgtggcaatgtgaactgaagctgatgggctgagaacatggactgagcttgtggtgtgctttgcaggaggacttgaagcagagttcaccagtgagctcaggtgtctcaaagaagggtggaagttctaatgtctgttagctacccataagaatgctgtttgctgcagttctgtgtcctgtgcttggatgctttttataagagttgtcattgttggaaattcttaaataaaactgatttaaataatatgtgtctttgttttgcagccctgaatgcaaagaattcatagcagttaattccccttttttgacccttttgagatggaactttcataaagtttcttggcagtagtttattttgcttcaaataaacttatttga

SEQ ID NO: 19 - DNA, 681 bp, synthetic construct
  misc_feature 1..681: note = synthesized nucleotides
  source 1..681: mol_type = other DNA
atgaacaaaagaaaaatggatgagacagatgcttcatcagcagtgaaagtgaaaagagcagtccagaaaacatccgatttaatagtgttgggtctcccatggaaaacaaccgaacaggacctgaaagagtattttagtacctttggagaagttcttatggtgcaggtcaagaaagatcttaagactggtcattcaaaggggtttggctttgttcgttttacggaatatgaaacacaagtgaaagtaatgtcacagcgacatatgatagatggacgatggtgtgactgcaaacttcctaattctaagcaaagccaagatgagcctttgagaagcagaaaagtgtttgtggggcgctgtacagaggacatgactgaggatgagctgcgggagttcttctctcagtacggggatgtgatggatgtcttcatccccaagccattcagggcctttgcctttgttacatttgcagatgatcagattgcgcagtctctttgtggagaggacttgatcattaaaggaatcagcgttcatatatccaatgccgaacctaagcacaatagcaatagacagttagaaagaagtggaagatttggtgttcatctcatttcaaatgtttatggaagaagcacttcattgaaagtagtgctggaacaaaaactcatctcagaagaggatctgtag

SEQ ID NO: 20 - DNA, 21 bp, synthetic construct
  misc_feature 1..21: note = synthesized nucleotides
  source 1..21: mol_type = other DNA
aggaagagctaaaggaatttt

SEQ ID NO: 21 - DNA, 1679 bp, artificial
  source 1..1679: mol_type = other DNA
atggtgagcaagggcgaggagctgttcaccggggtggtgcccatcctggtcgagctggacggcgacgtaaacggccacaagttcagcgtgtccggcgagggcgagggcgatgccacctacggcaagctgaccctgaagttcatctgcaccaccggcaagctgcccgtgccctggcccaccctcgtgaccaccctgacctacggcgtgcagtgcttcagccgctaccccgaccacatgaagcagcacgacttcttcaagtccgccatgcccgaaggctacgtccaggagcgcaccatcttcttcaaggacgacggcaactacaagacccgcgccgaggtgaagttcgagggcgacaccctggtgaaccgcatcgagctgaagggcatcgacttcaaggaggacggcaacatcctggggcacaagctggagtacaactacaacagccacaacgtctatatcatggccgacaagcagaagaacggcatcaaggtgaacttcaagatccgccacaacatcgaggacggcagcgtgcagctcgccgaccactaccagcagaacacccccatcggcgacggccccgtgctgctgcccgacaaccactacctgagcacccagtccgccctgagcaaagaccccaacgagaagcgcgatcacatggtcctgctggagttcgtgaccgccgccgggatcactctcggcatggacgagctgtacaagtaaatattctgccataggaatactgtctacatgctttctcattcaagaattcgtcatcacgcatcacaggccgcgtctttgacggtgggtgtcccatttttatccgctactctttatttcatggagtcgtatcaacgctatgaacgcaaggctgtgatatggaaccagaaggctgtctgaacttttgaaaccttgtgtgtgtgtgtgtgtgggattgatggtggtgccgaggcatgaaaggctagtatgagcgagaaaaggagagagcgcgtgcagagacttggtggtgcataatggatattttttaacttggcgagatgtgtctctcaatcctgtggctttggtgagagagtgtgtgtgtgtgtgcagagagcaatgatagcaaataatgtacgaatgttttttgcattcaaaggacatccacatctgttggaagacttttaagtgagtttttgttcttagataacccacattagatgaatgtgttaagtgaaatgatacttgtactccccctacccctttgtcaactgctgtgaatgctgtatggtgtgtgtgtgtgtgttctcttctgttactgatatgtaagtgtggcaatgtgaactgaagctgatgggctgagaacatggactgagcttgtggtgtgctttgcaggaggacttgaagcagagttcaccagtgagctcaggtgtctcaaagaagggtggaagttctaatgtctgttagctacccataagaatgctgtttgctgcagttctgtgtcctgtgcttggatgctttttataagagttgtcattgttggaaattcttaaataaaactgatttaaataatatgtgtctttgttttgcagccctgaatgcaaagaattcatagcagttaattccccttttttgacccttttgagatggaactttcataaagtttcttggcagtagtttattttgcttcaaataaacttatttga